European Patent Application EP 4 813 400 A1, published September 30, 2026. Title: Miscela comprendente ceppi probiotici e vitamina D, composizione e loro uso medico. Applicant: Beingpharma S.r.l. Application EP. The sequence listing filed with the application follows.

SEQUENCE LISTING (2 sequences)

SEQ ID NO: 1 - DNA, 17 bp, synthetic construct
  source 1..17: mol_type = other DNA
cctacgggnbgcascag

SEQ ID NO: 2 - DNA, 21 bp, synthetic construct
  source 1..21: mol_type = other DNA
gactacnvgggtatctaatcc